European Patent Application EP 4 660 192 A1, published December 10, 2025. Title: SALT INDUCIBLE KINASE INHIBITORS. Applicant: THE GENERAL HOSPITAL CORPORATION. Application IB PCT/US2021/044673, filed August 5, 2021. The sequence listing filed with the application follows.

SEQUENCE LISTING (6 sequences)

SEQ ID NO: 1 - DNA, 20 bp, synthetic construct
  misc_feature 1..20: note = synthetic primer
  source 1..20: mol_type = other DNA
cctctatgccaacacagtgc

SEQ ID NO: 2 - DNA, 20 bp, synthetic construct
  misc_feature 1..20: note = synthetic primer
  source 1..20: mol_type = other DNA
acatctgctggaaggtggac

SEQ ID NO: 3 - DNA, 20 bp, synthetic construct
  misc_feature 1..20: note = synthetic primer
  source 1..20: mol_type = other DNA
gcctcatctgcctacttgtg

SEQ ID NO: 4 - DNA, 20 bp, synthetic construct
  misc_feature 1..20: note = synthetic primer
  source 1..20: mol_type = other DNA
ctgtggcatcattcctgaag

SEQ ID NO: 5 - DNA, 20 bp, synthetic construct
  misc_feature 1..20: note = synthetic primer
  source 1..20: mol_type = other DNA
gctgggccaagatctctaac

SEQ ID NO: 6 - DNA, 20 bp, synthetic construct
  misc_feature 1..20: note = synthetic primer
  source 1..20: mol_type = other DNA
gtaggtacgcttcccgatgt